European Patent Application EP 4 481 033 A1, published December 25, 2024. Title: Microorganism producing L-amino acid with weakened activity of carbamoyl-phosphate synthetase and L-amino acid production method using the same. Applicant: CJ CheilJedang Corporation. The sequence listing filed with the application follows.

SEQUENCE LISTING (28 sequences)

SEQ ID NO: 1 - protein, 393 aa, unidentified
  REGION 1..393: note = CarA
MSKDTTTYQGVTEIGSVPAYLVLADGRTFTGFGFGAIGTTLGEAVFTTAMTGYQETMTDPSYHRQIVVATAPQIGNTGWNDEDNESRDGKIWVAGLVIRDLAARVSNWRATTSLQQEMADQGIVGIGGIDTRALVRHLRNEGSIAAGIFSGADAQRPVEELVEIVKNQPAMTGANLSVEVSADETYVIEAEGEERHTVVAYDLGIKQNTPRRFSARGVRTVIVPAETPLEDIKQYNPSGVFISNGPGDPAAADVMVDIVREVLEADIPFFGICFGNQILGRAFGMETYKLKFGHRGINVPVKNHITGKIDITAQNHGFALKGEAGQEFETDFGTAIVTHTCLNDGVVEGVALKSGRAYSVQYHPEAAAGPNDASPLFDQFVELMDADAQKKGA

SEQ ID NO: 2 - protein, 1113 aa, unidentified
  REGION 1..1113: note = CarAB
MPKRSDINHVLVIGSGPIVIGQACEFDYSGTQACRVLKEEGLRVTLINSNPATIMTDPEMADHTYVEPIEPEYIDKIFAKEIEQGHPIDAVLATLGGQTALNAAIQLDRLGILEKYGVELIGADIDAIERGEDRQKFKDIVTTIGGESARSRVCHNMDEVHETVAELGLPVVVRPSFTMGGLGSGLAYNTEDLERIAGGGLAASPEANVLIEESILGWKEFELELMRDTADNVVVICSIENVDALGVHTGDSVTVAPALTLTDREFQKMRDQGIAIIREVGVDTGGCNIQFAINPVDGRIITIEMNPRVSRSSALASKATGFPIAKMAAKLAIGYTLDEITNDITGETPAAFEPTIDYVVVKAPRFAFEKFVGADDTLTTTMKSVGEVMSLGRNYIAALNKALRSLETKQQGFWTKPDEFFAGERATDKAAVLEDLKRPTEGRLYDVELAMRLGASVEELYEASSIDPWFLAELEALVQFRQKLVDAPFLNEDLLREAKFMGLSDLQIAALRPEFAGEDGVRTLRLSLGIRPVFKTVDTCAAEFEAKTPYHYSAYELDPAAESEVAPQTEREKVLILGSGPNRIGQGIEFDYSCVHAALELSRVGYETVMVNCNPETVSTDYDTADRLYFEPLTFEDVMEVYHAEAQSGTVAGVIVQLGGQTPLGLADRLKKAGVPVIGTSPEAIDMAEDRGEFGALLNREQLPAPAFGTATSFEEARTVADEISYPVLVRPSYVLGGRGMEIVYDEASLEDYINRATELSSDHPVLVDRFLDNAIEIDVDALCDGDEVYLAGVMEHIEEAGIHSGDSACALPPMTLGAQDIEKVREATKKLALGIGVQGLMNVQYALKDDILYVIEANPRASRTVPFVSKATGVNLAKAASRIAVGATIKDLQDEGMIPTEYDGGSLPLDAPIAVKEAVLPFNRFRRPDGKTLDTLLSPEMKSTGEVMGLANNFGAAYAKAEAGAFGALPTEGTVFVTVANRDKRTLILPIQRLASMGYKILATEGTAGMLRRNGIDCEVVLKASDIREGVEGKSIVDRIREGEVDLILNTPAGSAGARHDGYDIRAAAVTVGVPLITTVQGVTAAVQGIEALREGVVSVRALQELDHAVKA

SEQ ID NO: 3 - DNA, 4529 bp, unidentified
  misc_feature 1..4529: note = carAB
  source 1..4529: mol_type = genomic DNA
gtgagtaaagacaccaccacctaccagggagtcaccgagatcggatccgttccggcatacctggttcttgcagacggacgtaccttcaccggatttggctttggagctatcggcaccacccttggtgaggcagtgttcaccaccgccatgaccggttaccaagaaaccatgaccgatccttcctatcaccgccagattgttgtggctaccgcaccacagatcggtaacaccggctggaacgatgaggacaacgagtcccgcgacggcaagatttgggttgcaggccttgttatccgcgacctcgcagcacgtgtgtccaactggcgcgccaccacctccttgcagcaggaaatggcagaccaaggcatcgtcggcatcggcggaatcgacacccgcgcactggttcgccacctgcgcaacgaaggttccatcgcagcgggcatcttctccggcgctgacgcacagcgcccagttgaagaactcgtagagatcgtcaagaatcagccagcaatgaccggcgcaaacctctccgttgaggtctctgctgatgaaacctacgtcatcgaagctgagggcgaagagcgccacaccgtcgtggcctacgacctgggcattaagcaaaacaccccacgtcgtttctctgcacgcggtgttcgcaccgtcatcgtgcctgctgaaaccccattggaggacatcaagcagtacaacccatcaggcgtgtttatctccaatggccctggcgaccctgcagcagcagacgtcatggttgatatcgtccgcgaagttctggaagccgacattccattctttggcatctgcttcggcaaccagatcctcggccgcgcattcggcatggagacctacaagctgaagttcggccaccgcggcatcaacgttccagtgaagaaccacatcaccggcaagatcgacatcaccgcccagaaccacggcttcgcactcaagggtgaagcaggccaggaattcgagacagatttcggcactgcgattgtcacccacacctgccttaacgacggcgtcgttgaaggtgttgcgctgaagtccggacgcgcatactccgttcagtaccacccagaggccgctgccggcccaaatgatgcaagccccctgtttgaccagtttgttgagctgatggatgcagacgctcagaagaaaggcgcataaataacatgccaaagcgttcagatattaaccacgtcctcgtcatcggttccggccccatcgtcattggccaggcatgtgaattcgactactccggcacccaggcttgccgcgtgctgaaggaagagggactgcgcgtcaccctcatcaactccaacccagcaacgatcatgaccgacccagaaatggctgaccacacctacgtggagccaatcgagccggaatacatcgacaagattttcgctaaggagatcgagcagggccacccaatcgacgccgtcctggcaacccttggtggccagactgcacttaacgcagctatccagctggatcgcctcggcatcctggaaaagtacggcgttgaactcatcggtgcagacatcgatgccattgagcgcggcgaagatcgccagaagttcaaggatattgtcaccaccatcggtggcgaatccgcgcgttcccgcgtctgccacaacatggacgaagtccatgagactgtcgcagaacttggccttccagtagtcgtgcgtccatccttcactatgggtggcctgggctccggtcttgcatacaacaccgaagaccttgagcgcatcgcaggtggcggacttgctgcatctcctgaagcaaacgtcttgatcgaagaatccatccttggttggaaggaattcgagctcgagctcatgcgcgataccgcagacaacgttgtggttatctgctccattgaaaacgtcgacgcactgggcgtgcacaccggcgactctgtcaccgtggcacctgccctgaccctgactgaccgtgaattccagaagatgcgcgatcagggtatcgccatcatccgcgaggtcggcgtggacaccggtggatgtaacatccagttcgctatcaacccagttgatggccgcatcatcaccattgagatgaacccacgtgtgtctcgttcctccgcgctggcatccaaggcaacgggcttcccaattgccaagatggctgccaagctggctatcggatacaccctggatgagatcaccaacgacatcactggtgaaaccccagctgcgtttgagcccaccatcgactacgtcgtggtcaaggccccacgctttgctttcgagaagtttgtcggcgctgatgacactttgaccaccaccatgaagtccgtcggtgaggtcatgtccctgggccgtaactacattgcagcactgaacaaggcactgcgttccctggaaaccaagcagcagggtttctggaccaagcctgatgagttcttcgcaggggagcgcgctaccgataaggcagctgttctggaagatctcaagcgcccaaccgaaggccgcctctacgacgttgagctggcaatgcgccttggcgcaagcgtggaagaactctacgaagcatcttctattgatccttggttcctcgccgagcttgaagctctcgtgcagttccgccagaagctcgttgacgcaccattcctcaacgaagatctcctgcgcgaagcaaagttcatgggtctgtccgacctgcagatcgcagcccttcgcccagagttcgctggcgaagacggcgtacgcaccttgcgtctgtccctaggcatccgcccagtattcaagactgtggatacctgtgcagcagagtttgaagctaagactccgtaccactactccgcatacgagctggatccagcagctgagtctgaggtcgcaccacagactgagcgtgaaaaggtcctgatcttgggctccggtccaaaccgcatcggccagggcatcgagttcgactattcctgtgttcacgcagctcttgagctctcccgcgtcggctacgaaactgtcatggtcaactgcaacccagagaccgtgtccaccgactacgacaccgctgaccgcctgtacttcgagccactgaccttcgaagacgtcatggaggtctaccacgctgaggcgcagtccggcaccgtcgcaggtgttatcgtccagcttggtggccagactcctctgggcttggcagatcgtttgaagaaggctggcgtccctgtcattggtacctccccagaggcaatcgacatggctgaggaccgtggcgagttcggtgcactgctgaaccgcgagcagcttcctgctccagcattcggcaccgcaacctctttcgaagaggctcgcacagtagccgatgagatcagctacccagtgctggttcgcccttcctacgtcttgggtggccgtggcatggagattgtctacgatgaggcttccctcgaggattacatcaaccgcgcaactgagttgtcttctgaccacccagtgctggttgaccgcttcctggacaacgctattgagatcgacgtcgacgcactgtgcgacggcgacgaagtctacctggcgggcgtcatggaacacatcgaggaagccggcattcactccggtgactccgcatgtgcacttcctccaatgactttgggcgcacaggacatcgagaaggtccgcgaagcaaccaagaagctggctctgggcatcggcgtacagggcctgatgaacgtccagtacgcactcaaggacgacatcctctacgtcatcgaggcaaacccacgtgcatcccgcaccgtgccgttcgtctccaaggcaacgggcgtcaacctggccaaggcagcatcccgtatcgcagtgggcgccaccatcaaggatctccaagatgagggcatgattcctaccgagtacgacggcggctccttgccactggacgctccaatcgctgtgaaggaagcagtgttgccgttcaaccgcttccgtcgcccagatggaaagaccctggacaccctgctttccccagagatgaagtccactggcgaggtcatgggcttggccaacaacttcggcgctgcatatgcaaaggctgaagctggcgcgtttggtgcattgccaaccgaaggcaccgtcttcgtgaccgtggctaaccgcgacaagcgcaccctgatcctgccaatccagcgcctggcgtcgatgggctacaagatcctcgccaccgaaggcaccgcaggcatgctgcgccgcaacggcattgattgtgaagttgtgctcaaggcttccgacatccgcgaaggtgtagagggcaagtccatcgtggatcgtatccgcgaaggcgaagttgacctcatcctcaacaccccagctggttctgctggcgctcgccacgatggctacgatatccgcgcagcagcagtgaccgtgggtgttccactgatcaccactgtccagggtgtcaccgcagctgtccagggcattgaggccctgcgtgagggcgttgtcagcgtccgcgcgctgcaggaactcgaccacgcagtcaaggcttaa

SEQ ID NO: 4 - DNA, 400 bp, synthetic construct
  misc_feature 1..400: note = betP promoter
  source 1..400: mol_type = other DNA
ggcacaagatggggtgcgtggcgagatcaccgttgtcatcgaaggcgcgggcgatatcgcggtcgatgtcgattcgcttatcgacgccgcccagcagcgcgtcgattccggcgagcggttgaaagcggtgtgcgcagacctcgcgaaaatccatggcgtgagcaaaaatgaactctacgatgcggttatttctgccagggaaaattaatcgttatgtcattgtgatgctcccgtgaacataaacgggacctactggctttacttaagtaacagctatgtaaaagaccaggtcaggttcgggtcggtttaggtacgaaacccatttttcggtttgctttccaggtttccccaagtaaaggtgagttttatgactacatctgacccaaattcgaaaccgata

SEQ ID NO: 5 - DNA, 34 bp, synthetic construct
  misc_feature 1..34: note = primer 2
  source 1..34: mol_type = other DNA
ggcacaagatggggtgcgtggcgagatcaccgtt

SEQ ID NO: 6 - DNA, 34 bp, synthetic construct
  misc_feature 1..34: note = primer 3
  source 1..34: mol_type = other DNA
tatcggtttcgaatttgggtcagatgtagtcata

SEQ ID NO: 7 - DNA, 33 bp, synthetic construct
  misc_feature 1..33: note = primer 4
  source 1..33: mol_type = other DNA
cggtacccggggatcccaagaaggcgcttctcg

SEQ ID NO: 8 - DNA, 34 bp, synthetic construct
  misc_feature 1..34: note = primer 5
  source 1..34: mol_type = other DNA
gcaccccatcttgtgccggtgactgttgtcgcct

SEQ ID NO: 9 - DNA, 34 bp, synthetic construct
  misc_feature 1..34: note = primer 6
  source 1..34: mol_type = other DNA
caaattcgaaaccgatagtgagtaaagacaccac

SEQ ID NO: 10 - DNA, 33 bp, synthetic construct
  misc_feature 1..33: note = primer 7
  source 1..33: mol_type = other DNA
atgcctgcaggtcgacgagacctcaacggagag

SEQ ID NO: 11 - DNA, 20 bp, synthetic construct
  misc_feature 1..20: note = primer 8
  source 1..20: mol_type = other DNA
tattacgccagctggcgaaa

SEQ ID NO: 12 - DNA, 20 bp, synthetic construct
  misc_feature 1..20: note = primer 9
  source 1..20: mol_type = other DNA
gctttacactttatgcttcc

SEQ ID NO: 13 - DNA, 31 bp, synthetic construct
  misc_feature 1..31: note = primer 10
  source 1..31: mol_type = other DNA
ggtgactgttgtcgcctttcgtgtgtctgtc

SEQ ID NO: 14 - DNA, 33 bp, synthetic construct
  misc_feature 1..33: note = primer 11
  source 1..33: mol_type = other DNA
ggcgacaacagtcaccttgagtaaagacaccac

SEQ ID NO: 15 - DNA, 36 bp, synthetic construct
  misc_feature 1..36: note = primer 12
  source 1..36: mol_type = other DNA
cggtacccggggatcccccacgtcgtttctctgcac

SEQ ID NO: 16 - DNA, 21 bp, synthetic construct
  misc_feature 1..21: note = primer 13
  source 1..21: mol_type = other DNA
gttatttatgcgcctttcttc

SEQ ID NO: 17 - DNA, 38 bp, synthetic construct
  misc_feature 1..38: note = primer 14
  source 1..38: mol_type = other DNA
gaaaggcgcataaataacttgccaaagcgttcagatat

SEQ ID NO: 18 - DNA, 36 bp, synthetic construct
  misc_feature 1..36: note = primer 15
  source 1..36: mol_type = other DNA
atgcctgcaggtcgacgccacccatagtgaaggatg

SEQ ID NO: 19 - protein, 319 aa, unidentified
  REGION 1..319: note = ArgF
MTSQPQVRHFLADDDLTPAEQAEVLTLAAKLKAAPFSERPLEGPKSVAVLFDKTSTRTRFSFDAGIAHLGGHAIVVDSGSSQMGKGETLQDTAAVLSRYVEAIVWRTYAHSNFHAMAETSTVPLVNSLSDDLHPCQILADLQTIVENLSPEEGPAGLKGKKAVYLGDGDNNMANSYMIGFATAGMDISIIAPEGFQPRAEFVERAEKRGQETGAKVVVTDSLDEVAGADVVITDTWVSMGMENDGIDRTTPFVPYQVNDEVMAKANDGAIFLHCLPAYRGKEVAASVIDGPASKVFDEAENRLHAQKALLVWLLAHQPR

SEQ ID NO: 20 - DNA, 35 bp, synthetic construct
  misc_feature 1..35: note = primer 16
  source 1..35: mol_type = other DNA
cggtacccggggatcctgaccccaggcaagcacgg

SEQ ID NO: 21 - DNA, 27 bp, synthetic construct
  misc_feature 1..27: note = primer 17
  source 1..27: mol_type = other DNA
gaagcgagtacgagtttaagtcttatc

SEQ ID NO: 22 - DNA, 20 bp, synthetic construct
  misc_feature 1..20: note = primer 18
  source 1..20: mol_type = other DNA
aaactcgtactcgcttctcc

SEQ ID NO: 23 - DNA, 35 bp, synthetic construct
  misc_feature 1..35: note = primer 19
  source 1..35: mol_type = other DNA
atgcctgcaggtcgaccggcgccggcaacctcgtc

SEQ ID NO: 24 - protein, 171 aa, unidentified
  REGION 1..171: note = ArgR
MSLGSTPSTPENLNPVTRTARQALILQILDKQKVTSQVQLSELLLDEGIDITQATLSRDLDELGARKVRPDGGRAYYAVGPVDSIAREDLRGPSEKLRRMLDELLVSTDHSGNIAMLRTPPGAAQYLASFIDRVGLKEVVGTIAGDDTVFVLARDPLTGKELGELLSGRTT

SEQ ID NO: 25 - DNA, 36 bp, synthetic construct
  misc_feature 1..36: note = primer 20
  source 1..36: mol_type = other DNA
cggtacccggggatccctcgtgcggaattcgtggag

SEQ ID NO: 26 - DNA, 20 bp, synthetic construct
  misc_feature 1..20: note = primer 21
  source 1..20: mol_type = other DNA
atccagcagcaattcagaca

SEQ ID NO: 27 - DNA, 37 bp, synthetic construct
  misc_feature 1..37: note = primer 22
  source 1..37: mol_type = other DNA
ctgaattgctgctggattaaggcatcgatatcaccca

SEQ ID NO: 28 - DNA, 36 bp, synthetic construct
  misc_feature 1..36: note = primer 23
  source 1..36: mol_type = other DNA
atgcctgcaggtcgacccttcattttaagttccttg